European Patent Application EP 4 198 058 A1, published June 21, 2023. Title: Fusion protein comprising antibody for targeting oncogenic protein or single chain fragment variable (scFv) thereof and cancer cell penetrating peptide and use of the same. Applicant: NIBEC Co., Ltd. The sequence listing filed with the application follows.

SEQUENCE LISTING (93 sequences)

SEQ ID NO: 1 - protein, 271 aa, Artificial Sequence
  KRAS mutant scfv
MAWVWTLLFLMAAAQSIQAEWIKQRPGQGLEWIGVIHPGNGGTNYNENFKGKATLTADKSSSTAYMQLSSLTSDDSAVYFCASGNDGSYWGQGTTVTVSSGGGGSGKGGSGGGGSGGGGSDIELTQSPSSLTVTAGEKVTMSCKSSQSLLNSGDQKIYLTWYQQKPGQPPKLLIYWASTRESGVPDRFTGSVSGTDFTLTISSVQAEDLAVYYCQNDYNYPYTFGGGTKLEIKRGSENLYFQGGSGKPIPNPLLGLDSTGGSGGSHHHHHH

SEQ ID NO: 2 - protein, 254 aa, Artificial Sequence
  KRAS mutant scfv
MAQVKLQESGPELVRPGTSVKVSCKASGYAFTNYLIEWIKQRPGQGLEWIGVIHPGNGGTNYNENFKGKATLTADKSSSTAYMQLSSLTSDDSAVYFCASGNDGSYWGQGTTVTVSSGGGGSGGGGSGGGGSDIELTQSPSSLTVTAGEKVTMSCKSSQSLLNSGDQKIYLTWYQQKPGQPPKLLIYWASTRESGVPDRFTGSVSGTDFTLTISSVQAEDLAVYYCQNDYNYPYTFGGGTKLEIKRLEHHHHHH

SEQ ID NO: 3 - protein, 272 aa, Artificial Sequence
  KRAS mutant scfv
MAWVWTLLFLMAAAQSIQAEWIKQRPGQGLEWIGVIHPGNGGTNYNENFKGKATLTADKSSSTAYMQLSSLTSDDSAVYFCASGNDGSYWGQGTTVTVSSGGGGSGKGGSGGGGSGGGGSDIELTQSPSSLTVTAGEKVTMSCKSSQSLLNSGDQKIYLTWYQQKPGQPPKLLIYWASTRESGVPDRFTGSVSGTDFTLTISSVQAEDLAVYYCQNDYNYPYTFGGGTKCLEIKRGSENLYFQGGSGKPIPNPLLGLDSTGGSGGSHHHHHH

SEQ ID NO: 4 - protein, 16 aa, Artificial Sequence
  fusion peptide
GGGGSHRRCNKNNKKR

SEQ ID NO: 5 - protein, 16 aa, Artificial Sequence
  fusion peptide
GGGGSHRRCNPNNKKR

SEQ ID NO: 6 - protein, 19 aa, Artificial Sequence
  fusion peptide
GGGGSVSRRRRRRGGRRRR

SEQ ID NO: 7 - protein, 20 aa, Artificial Sequence
  fusion peptide
GGGGSGKCSTRGRKCCRRKK

SEQ ID NO: 8 - protein, 16 aa, Artificial Sequence
  fusion peptide
HRRCNKNNKKRGGGGS

SEQ ID NO: 9 - protein, 16 aa, Artificial Sequence
  fusion peptide
HRRCNPNNKKRGGGGS

SEQ ID NO: 10 - protein, 19 aa, Artificial Sequence
  fusion peptide
VSRRRRRRGGRRRRGGGGS

SEQ ID NO: 11 - protein, 20 aa, Artificial Sequence
  fusion peptide
GKCSTRGRKCCRRKKGGGGS

SEQ ID NO: 12 - protein, 287 aa, Artificial Sequence
  fusion peptide
MAWVWTLLFLMAAAQSIQAEWIKQRPGQGLEWIGVIHPGNGGTNYNENFKGKATLTADKSSSTAYMQLSSLTSDDSAVYFCASGNDGSYWGQGTTVTVSSGGGGSGKGGSGGGGSGGGGSDIELTQSPSSLTVTAGEKVTMSCKSSQSLLNSGDQKIYLTWYQQKPGQPPKLLIYWASTRESGVPDRFTGSVSGTDFTLTISSVQAEDLAVYYCQNDYNYPYTFGGGTKGGGGSHRRCNKNNKKRLEIKRGSENLYFQGGSGKPIPNPLLGLDSTGGSGGSHHHHHH

SEQ ID NO: 13 - protein, 287 aa, Artificial Sequence
  fusion peptide
MAWVWTLLFLMAAAQSIQAEWIKQRPGQGLEWIGVIHPGNGGTNYNENFKGKATLTADKSSSTAYMQLSSLTSDDSAVYFCASGNDGSYWGQGTTVTVSSGGGGSGKGGSGGGGSGGGGSDIELTQSPSSLTVTAGEKVTMSCKSSQSLLNSGDQKIYLTWYQQKPGQPPKLLIYWASTRESGVPDRFTGSVSGTDFTLTISSVQAEDLAVYYCQNDYNYPYTFGGGTKGGGGSHRRCNPNNKKRLEIKRGSENLYFQGGSGKPIPNPLLGLDSTGGSGGSHHHHHH

SEQ ID NO: 14 - protein, 290 aa, Artificial Sequence
  fusion peptide
MAWVWTLLFLMAAAQSIQAEWIKQRPGQGLEWIGVIHPGNGGTNYNENFKGKATLTADKSSSTAYMQLSSLTSDDSAVYFCASGNDGSYWGQGTTVTVSSGGGGSGKGGSGGGGSGGGGSDIELTQSPSSLTVTAGEKVTMSCKSSQSLLNSGDQKIYLTWYQQKPGQPPKLLIYWASTRESGVPDRFTGSVSGTDFTLTISSVQAEDLAVYYCQNDYNYPYTFGGGTKGGGGSVSRRRRRRGGRRRRLEIKRGSENLYFQGGSGKPIPNPLLGLDSTGGSGGSHHHHHH

SEQ ID NO: 15 - protein, 291 aa, Artificial Sequence
  fusion peptide
MAWVWTLLFLMAAAQSIQAEWIKQRPGQGLEWIGVIHPGNGGTNYNENFKGKATLTADKSSSTAYMQLSSLTSDDSAVYFCASGNDGSYWGQGTTVTVSSGGGGSGKGGSGGGGSGGGGSDIELTQSPSSLTVTAGEKVTMSCKSSQSLLNSGDQKIYLTWYQQKPGQPPKLLIYWASTRESGVPDRFTGSVSGTDFTLTISSVQAEDLAVYYCQNDYNYPYTFGGGTKGGGGSGKCSTRGRKCCRRKKLEIKRGSENLYFQGGSGKPIPNPLLGLDSTGGSGGSHHHHHH

SEQ ID NO: 16 - protein, 287 aa, Artificial Sequence
  fusion peptide
MAWVWTLLFLMAAAQSIQAHRRCNKNNKKRGGGGSEWIKQRPGQGLEWIGVIHPGNGGTNYNENFKGKATLTADKSSSTAYMQLSSLTSDDSAVYFCASGNDGSYWGQGTTVTVSSGGGGSGKGGSGGGGSGGGGSDIELTQSPSSLTVTAGEKVTMSCKSSQSLLNSGDQKIYLTWYQQKPGQPPKLLIYWASTRESGVPDRFTGSVSGTDFTLTISSVQAEDLAVYYCQNDYNYPYTFGGGTKLEIKRGSENLYFQGGSGKPIPNPLLGLDSTGGSGGSHHHHHH

SEQ ID NO: 17 - protein, 287 aa, Artificial Sequence
  fusion peptide
MAWVWTLLFLMAAAQSIQAHRRCNPNNKKRGGGGSEWIKQRPGQGLEWIGVIHPGNGGTNYNENFKGKATLTADKSSSTAYMQLSSLTSDDSAVYFCASGNDGSYWGQGTTVTVSSGGGGSGKGGSGGGGSGGGGSDIELTQSPSSLTVTAGEKVTMSCKSSQSLLNSGDQKIYLTWYQQKPGQPPKLLIYWASTRESGVPDRFTGSVSGTDFTLTISSVQAEDLAVYYCQNDYNYPYTFGGGTKLEIKRGSENLYFQGGSGKPIPNPLLGLDSTGGSGGSHHHHHH

SEQ ID NO: 18 - protein, 290 aa, Artificial Sequence
  fusion peptide
MAWVWTLLFLMAAAQSIQAVSRRRRRRGGRRRRGGGGSEWIKQRPGQGLEWIGVIHPGNGGTNYNENFKGKATLTADKSSSTAYMQLSSLTSDDSAVYFCASGNDGSYWGQGTTVTVSSGGGGSGKGGSGGGGSGGGGSDIELTQSPSSLTVTAGEKVTMSCKSSQSLLNSGDQKIYLTWYQQKPGQPPKLLIYWASTRESGVPDRFTGSVSGTDFTLTISSVQAEDLAVYYCQNDYNYPYTFGGGTKLEIKRGSENLYFQGGSGKPIPNPLLGLDSTGGSGGSHHHHHH

SEQ ID NO: 19 - protein, 291 aa, Artificial Sequence
  fusion peptide
MAWVWTLLFLMAAAQSIQAGKCSTRGRKCCRRKKGGGGSEWIKQRPGQGLEWIGVIHPGNGGTNYNENFKGKATLTADKSSSTAYMQLSSLTSDDSAVYFCASGNDGSYWGQGTTVTVSSGGGGSGKGGSGGGGSGGGGSDIELTQSPSSLTVTAGEKVTMSCKSSQSLLNSGDQKIYLTWYQQKPGQPPKLLIYWASTRESGVPDRFTGSVSGTDFTLTISSVQAEDLAVYYCQNDYNYPYTFGGGTKLEIKRGSENLYFQGGSGKPIPNPLLGLDSTGGSGGSHHHHHH

SEQ ID NO: 20 - protein, 270 aa, Artificial Sequence
  fusion peptide
MAQVKLQESGPELVRPGTSVKVSCKASGYAFTNYLIEWIKQRPGQGLEWIGVIHPGNGGTNYNENFKGKATLTADKSSSTAYMQLSSLTSDDSAVYFCASGNDGSYWGQGTTVTVSSGGGGSGGGGSGGGGSDIELTQSPSSLTVTAGEKVTMSCKSSQSLLNSGDQKIYLTWYQQKPGQPPKLLIYWASTRESGVPDRFTGSVSGTDFTLTISSVQAEDLAVYYCQNDYNYPYTFGGGTKGGGGSHRRCNKNNKKRLEIKRLEHHHHHH

SEQ ID NO: 21 - protein, 270 aa, Artificial Sequence
  fusion peptide
MAQVKLQESGPELVRPGTSVKVSCKASGYAFTNYLIEWIKQRPGQGLEWIGVIHPGNGGTNYNENFKGKATLTADKSSSTAYMQLSSLTSDDSAVYFCASGNDGSYWGQGTTVTVSSGGGGSGGGGSGGGGSDIELTQSPSSLTVTAGEKVTMSCKSSQSLLNSGDQKIYLTWYQQKPGQPPKLLIYWASTRESGVPDRFTGSVSGTDFTLTISSVQAEDLAVYYCQNDYNYPYTFGGGTKGGGGSHRRCNPNNKKRLEIKRLEHHHHHH

SEQ ID NO: 22 - protein, 273 aa, Artificial Sequence
  fusion peptide
MAQVKLQESGPELVRPGTSVKVSCKASGYAFTNYLIEWIKQRPGQGLEWIGVIHPGNGGTNYNENFKGKATLTADKSSSTAYMQLSSLTSDDSAVYFCASGNDGSYWGQGTTVTVSSGGGGSGGGGSGGGGSDIELTQSPSSLTVTAGEKVTMSCKSSQSLLNSGDQKIYLTWYQQKPGQPPKLLIYWASTRESGVPDRFTGSVSGTDFTLTISSVQAEDLAVYYCQNDYNYPYTFGGGTKGGGGSVSRRRRRRGGRRRRLEIKRLEHHHHHH

SEQ ID NO: 23 - protein, 274 aa, Artificial Sequence
  fusion peptide
MAQVKLQESGPELVRPGTSVKVSCKASGYAFTNYLIEWIKQRPGQGLEWIGVIHPGNGGTNYNENFKGKATLTADKSSSTAYMQLSSLTSDDSAVYFCASGNDGSYWGQGTTVTVSSGGGGSGGGGSGGGGSDIELTQSPSSLTVTAGEKVTMSCKSSQSLLNSGDQKIYLTWYQQKPGQPPKLLIYWASTRESGVPDRFTGSVSGTDFTLTISSVQAEDLAVYYCQNDYNYPYTFGGGTKGGGGSGKCSTRGRKCCRRKKLEIKRLEHHHHHH

SEQ ID NO: 24 - protein, 275 aa, Artificial Sequence
  fusion peptide
MAQVKLQESGPELVRPGTSVKVSCKASGYAFTNYLIHRRCNKNNKKRGGGGSEWIKQRPGQGLEWIGVIHPGNGGTNYNENFKGKATLTADKSSSTAYMQLSSLTSDDSAVYFCASGNDGSYWGQGTTVTVSSGGGGSGKGGSGGGGSGGGGSDIELTQSPSSLTVTAGEKVTMSCKSSQSLLNSGDQKIYLTWYQQKPGQPPKLLIYWASTRESGVPDRFTGSVSGTDFTLTISSVQAEDLAVYYCQNDYNYPYTFGGGTKLEIKRLEHHHHHH

SEQ ID NO: 25 - protein, 275 aa, Artificial Sequence
  fusion peptide
MAQVKLQESGPELVRPGTSVKVSCKASGYAFTNYLIHRRCNPNNKKRGGGGSEWIKQRPGQGLEWIGVIHPGNGGTNYNENFKGKATLTADKSSSTAYMQLSSLTSDDSAVYFCASGNDGSYWGQGTTVTVSSGGGGSGKGGSGGGGSGGGGSDIELTQSPSSLTVTAGEKVTMSCKSSQSLLNSGDQKIYLTWYQQKPGQPPKLLIYWASTRESGVPDRFTGSVSGTDFTLTISSVQAEDLAVYYCQNDYNYPYTFGGGTKLEIKRLEHHHHHH

SEQ ID NO: 26 - protein, 278 aa, Artificial Sequence
  fusion peptide
MAQVKLQESGPELVRPGTSVKVSCKASGYAFTNYLIVSRRRRRRGGRRRRGGGGSEWIKQRPGQGLEWIGVIHPGNGGTNYNENFKGKATLTADKSSSTAYMQLSSLTSDDSAVYFCASGNDGSYWGQGTTVTVSSGGGGSGKGGSGGGGSGGGGSDIELTQSPSSLTVTAGEKVTMSCKSSQSLLNSGDQKIYLTWYQQKPGQPPKLLIYWASTRESGVPDRFTGSVSGTDFTLTISSVQAEDLAVYYCQNDYNYPYTFGGGTKLEIKRLEHHHHHH

SEQ ID NO: 27 - protein, 280 aa, Artificial Sequence
  fusion peptide
MAQVKLQESGPELVRPGTSVKVSCKASGYAFTNYLIGKCSTRGRKCCRRKKGGGGSEWIKQRPGQGLEWIGVIHPGNGGTNYNENFKGKATLTADKSSSTAYMQLSSLTSDDSAVYFCASGNDGSYWGQGTTVTVSSGGGGSGKGGSGGGGSGGGGSDIELTQSPSSLTVTAGEKVTMSCKSSQSLLNSGDQKIYLTWYQQKPGQPPKLLIYWASTRESGVPDRFTGSVSGTDFTLTISSVQAEDLAVYYCQNDYNYPYTFGGGTKLEIKRLEHHHHHHH

SEQ ID NO: 28 - protein, 287 aa, Artificial Sequence; identical to SEQ ID NO: 12
  fusion peptide

SEQ ID NO: 29 - protein, 287 aa, Artificial Sequence; identical to SEQ ID NO: 13
  fusion peptide

SEQ ID NO: 30 - protein, 290 aa, Artificial Sequence; identical to SEQ ID NO: 14
  fusion peptide

SEQ ID NO: 31 - protein, 291 aa, Artificial Sequence; identical to SEQ ID NO: 15
  fusion peptide

SEQ ID NO: 32 - protein, 287 aa, Artificial Sequence; identical to SEQ ID NO: 16
  fusion peptide

SEQ ID NO: 33 - protein, 287 aa, Artificial Sequence; identical to SEQ ID NO: 17
  fusion peptide

SEQ ID NO: 34 - protein, 290 aa, Artificial Sequence; identical to SEQ ID NO: 18
  fusion peptide

SEQ ID NO: 35 - protein, 291 aa, Artificial Sequence; identical to SEQ ID NO: 19
  fusion peptide

SEQ ID NO: 36 - protein, 270 aa, Artificial Sequence; identical to SEQ ID NO: 20
  fusion peptide

SEQ ID NO: 37 - protein, 270 aa, Artificial Sequence; identical to SEQ ID NO: 21
  fusion peptide

SEQ ID NO: 38 - protein, 273 aa, Artificial Sequence; identical to SEQ ID NO: 22
  fusion peptide

SEQ ID NO: 39 - protein, 274 aa, Artificial Sequence; identical to SEQ ID NO: 23
  fusion peptide

SEQ ID NO: 40 - protein, 275 aa, Artificial Sequence; identical to SEQ ID NO: 24
  fusion peptide

SEQ ID NO: 41 - protein, 275 aa, Artificial Sequence; identical to SEQ ID NO: 25
  fusion peptide

SEQ ID NO: 42 - protein, 278 aa, Artificial Sequence; identical to SEQ ID NO: 26
  fusion peptide

SEQ ID NO: 43 - protein, 280 aa, Artificial Sequence; identical to SEQ ID NO: 27
  fusion peptide

SEQ ID NO: 44 - protein, 287 aa, Artificial Sequence; identical to SEQ ID NO: 12
  fusion peptide

SEQ ID NO: 45 - protein, 287 aa, Artificial Sequence; identical to SEQ ID NO: 13
  fusion peptide

SEQ ID NO: 46 - protein, 290 aa, Artificial Sequence; identical to SEQ ID NO: 14
  fusion peptide

SEQ ID NO: 47 - protein, 291 aa, Artificial Sequence; identical to SEQ ID NO: 15
  fusion peptide

SEQ ID NO: 48 - protein, 287 aa, Artificial Sequence; identical to SEQ ID NO: 16
  fusion peptide

SEQ ID NO: 49 - protein, 287 aa, Artificial Sequence; identical to SEQ ID NO: 17
  fusion peptide

SEQ ID NO: 50 - protein, 290 aa, Artificial Sequence; identical to SEQ ID NO: 18
  fusion peptide

SEQ ID NO: 51 - protein, 291 aa, Artificial Sequence; identical to SEQ ID NO: 19
  fusion peptide

SEQ ID NO: 52 - protein, 270 aa, Artificial Sequence; identical to SEQ ID NO: 20
  fusion peptide

SEQ ID NO: 53 - protein, 270 aa, Artificial Sequence; identical to SEQ ID NO: 21
  fusion peptide

SEQ ID NO: 54 - protein, 273 aa, Artificial Sequence; identical to SEQ ID NO: 22
  fusion peptide

SEQ ID NO: 55 - protein, 274 aa, Artificial Sequence; identical to SEQ ID NO: 23
  fusion peptide

SEQ ID NO: 56 - protein, 275 aa, Artificial Sequence; identical to SEQ ID NO: 24
  fusion peptide

SEQ ID NO: 57 - protein, 275 aa, Artificial Sequence; identical to SEQ ID NO: 25
  fusion peptide

SEQ ID NO: 58 - protein, 278 aa, Artificial Sequence; identical to SEQ ID NO: 26
  fusion peptide

SEQ ID NO: 59 - protein, 280 aa, Artificial Sequence; identical to SEQ ID NO: 27
  fusion peptide

SEQ ID NO: 60 - protein, 17 aa, Artificial Sequence
  fusion peptide
CGGGGGHRRCNKNNKKR

SEQ ID NO: 61 - protein, 17 aa, Artificial Sequence
  fusion peptide
CGGGGGHRRCNPNNKKR

SEQ ID NO: 62 - protein, 20 aa, Artificial Sequence
  fusion peptide
CGGGGGVSRRRRRRGGRRRR

SEQ ID NO: 63 - protein, 21 aa, Artificial Sequence
  fusion peptide
CGGGGGGKCSTRGRKCCRRKK

SEQ ID NO: 64 - protein, 24 aa, Artificial Sequence
  fusion peptide
CGGGGGSSGGGGGRKKNNKNCRRH

SEQ ID NO: 65 - protein, 24 aa, Artificial Sequence
  fusion peptide
CGGGGGSSGGGGGRKKNNPNCRRH

SEQ ID NO: 66 - protein, 27 aa, Artificial Sequence
  fusion peptide
CGGGGGSSGGGGGRRRRGGRRRRRRSV

SEQ ID NO: 67 - protein, 28 aa, Artificial Sequence
  fusion peptide
CGGGGGSSGGGGGGKCSTRGRKCCRRKK

SEQ ID NO: 68 - protein, 288 aa, Artificial Sequence
  fusion peptide
MAWVWTLLFLMAAAQSIQAEWIKQRPGQGLEWIGVIHPGNGGTNYNENFKGKATLTADKSSSTAYMQLSSLTSDDSAVYFCASGNDGSYWGQGTTVTVSSGGGGSGKCGGGGGHRRCNKNNKKRGGSGGGGSGGGGSDIELTQSPSSLTVTAGEKVTMSCKSSQSLLNSGDQKIYLTWYQQKPGQPPKLLIYWASTRESGVPDRFTGSVSGTDFTLTISSVQAEDLAVYYCQNDYNYPYTFGGGTKLEIKRGSENLYFQGGSGKPIPNPLLGLDSTGGSGGSHHHHHH

SEQ ID NO: 69 - protein, 288 aa, Artificial Sequence
  fusion peptide
MAWVWTLLFLMAAAQSIQAEWIKQRPGQGLEWIGVIHPGNGGTNYNENFKGKATLTADKSSSTAYMQLSSLTSDDSAVYFCASGNDGSYWGQGTTVTVSSGGGGSGKCGGGGGHRRCNPNNKKRGGSGGGGSGGGGSDIELTQSPSSLTVTAGEKVTMSCKSSQSLLNSGDQKIYLTWYQQKPGQPPKLLIYWASTRESGVPDRFTGSVSGTDFTLTISSVQAEDLAVYYCQNDYNYPYTFGGGTKLEIKRGSENLYFQGGSGKPIPNPLLGLDSTGGSGGSHHHHHH

SEQ ID NO: 70 - protein, 291 aa, Artificial Sequence
  fusion peptide
MAWVWTLLFLMAAAQSIQAEWIKQRPGQGLEWIGVIHPGNGGTNYNENFKGKATLTADKSSSTAYMQLSSLTSDDSAVYFCASGNDGSYWGQGTTVTVSSGGGGSGKCGGGGGVSRRRRRRGGRRRRGGSGGGGSGGGGSDIELTQSPSSLTVTAGEKVTMSCKSSQSLLNSGDQKIYLTWYQQKPGQPPKLLIYWASTRESGVPDRFTGSVSGTDFTLTISSVQAEDLAVYYCQNDYNYPYTFGGGTKLEIKRGSENLYFQGGSGKPIPNPLLGLDSTGGSGGSHHHHHH

SEQ ID NO: 71 - protein, 292 aa, Artificial Sequence
  fusion peptide
MAWVWTLLFLMAAAQSIQAEWIKQRPGQGLEWIGVIHPGNGGTNYNENFKGKATLTADKSSSTAYMQLSSLTSDDSAVYFCASGNDGSYWGQGTTVTVSSGGGGSGKCGGGGGGKCSTRGRKCCRRKKGGSGGGGSGGGGSDIELTQSPSSLTVTAGEKVTMSCKSSQSLLNSGDQKIYLTWYQQKPGQPPKLLIYWASTRESGVPDRFTGSVSGTDFTLTISSVQAEDLAVYYCQNDYNYPYTFGGGTKLEIKRGSENLYFQGGSGKPIPNPLLGLDSTGGSGGSHHHHHH

SEQ ID NO: 72 - protein, 294 aa, Artificial Sequence
  fusion peptide
MAWVWTLLFLMAAAQSIQAEWIKQRPGQGLEWIGVIHPGNGGTNYNENFKGKATLTADKSSSTAYMQLSSLTSDDSAVYFCASGNDGSYWGQGTTVTVSSGGGGSGKCGGGGGSSGGGGHRRCNKNNKKRGGSGGGGSGGGGSDIELTQSPSSLTVTAGEKVTMSCKSSQSLLNSGDQKIYLTWYQQKPGQPPKLLIYWASTRESGVPDRFTGSVSGTDFTLTISSVQAEDLAVYYCQNDYNYPYTFGGGTKLEIKRGSENLYFQGGSGKPIPNPLLGLDSTGGSGGSHHHHHH

SEQ ID NO: 73 - protein, 295 aa, Artificial Sequence
  fusion peptide
MAWVWTLLFLMAAAQSIQAEWIKQRPGQGLEWIGVIHPGNGGTNYNENFKGKATLTADKSSSTAYMQLSSLTSDDSAVYFCASGNDGSYWGQGTTVTVSSGGGGSGKCGGGGGSSGGGGGRKKNNPNCRRHGGSGGGGSGGGGSDIELTQSPSSLTVTAGEKVTMSCKSSQSLLNSGDQKIYLTWYQQKPGQPPKLLIYWASTRESGVPDRFTGSVSGTDFTLTISSVQAEDLAVYYCQNDYNYPYTFGGGTKLEIKRGSENLYFQGGSGKPIPNPLLGLDSTGGSGGSHHHHHH

SEQ ID NO: 74 - protein, 298 aa, Artificial Sequence
  fusion peptide
MAWVWTLLFLMAAAQSIQAEWIKQRPGQGLEWIGVIHPGNGGTNYNENFKGKATLTADKSSSTAYMQLSSLTSDDSAVYFCASGNDGSYWGQGTTVTVSSGGGGSGKCGGGGGSSGGGGGRRRRGGRRRRRRSVGGSGGGGSGGGGSDIELTQSPSSLTVTAGEKVTMSCKSSQSLLNSGDQKIYLTWYQQKPGQPPKLLIYWASTRESGVPDRFTGSVSGTDFTLTISSVQAEDLAVYYCQNDYNYPYTFGGGTKLEIKRGSENLYFQGGSGKPIPNPLLGLDSTGGSGGSHHHHHH

SEQ ID NO: 75 - protein, 299 aa, Artificial Sequence
  fusion peptide
MAWVWTLLFLMAAAQSIQAEWIKQRPGQGLEWIGVIHPGNGGTNYNENFKGKATLTADKSSSTAYMQLSSLTSDDSAVYFCASGNDGSYWGQGTTVTVSSGGGGSGKCGGGGGSSGGGGGGKCSTRGRKCCRRKKGGSGGGGSGGGGSDIELTQSPSSLTVTAGEKVTMSCKSSQSLLNSGDQKIYLTWYQQKPGQPPKLLIYWASTRESGVPDRFTGSVSGTDFTLTISSVQAEDLAVYYCQNDYNYPYTFGGGTKLEIKRGSENLYFQGGSGKPIPNPLLGLDSTGGSGGSHHHHHH

SEQ ID NO: 76 - protein, 289 aa, Artificial Sequence
  fusion peptide
MAWVWTLLFLMAAAQSIQAEWIKQRPGQGLEWIGVIHPGNGGTNYNENFKGKATLTADKSSSTAYMQLSSLTSDDSAVYFCASGNDGSYWGQGTTVTVSSGGGGSGKGGSGGGGSGGGGSDIELTQSPSSLTVTAGEKVTMSCKSSQSLLNSGDQKIYLTWYQQKPGQPPKLLIYWASTRESGVPDRFTGSVSGTDFTLTISSVQAEDLAVYYCQNDYNYPYTFGGGTKCCGGGGGHRRCNKNNKKRLEIKRGSENLYFQGGSGKPIPNPLLGLDSTGGSGGSHHHHHH

SEQ ID NO: 77 - protein, 289 aa, Artificial Sequence
  fusion peptide
MAWVWTLLFLMAAAQSIQAEWIKQRPGQGLEWIGVIHPGNGGTNYNENFKGKATLTADKSSSTAYMQLSSLTSDDSAVYFCASGNDGSYWGQGTTVTVSSGGGGSGKGGSGGGGSGGGGSDIELTQSPSSLTVTAGEKVTMSCKSSQSLLNSGDQKIYLTWYQQKPGQPPKLLIYWASTRESGVPDRFTGSVSGTDFTLTISSVQAEDLAVYYCQNDYNYPYTFGGGTKCCGGGGGHRRCNPNNKKRLEIKRGSENLYFQGGSGKPIPNPLLGLDSTGGSGGSHHHHHH

SEQ ID NO: 78 - protein, 292 aa, Artificial Sequence
  fusion peptide
MAWVWTLLFLMAAAQSIQAEWIKQRPGQGLEWIGVIHPGNGGTNYNENFKGKATLTADKSSSTAYMQLSSLTSDDSAVYFCASGNDGSYWGQGTTVTVSSGGGGSGKGGSGGGGSGGGGSDIELTQSPSSLTVTAGEKVTMSCKSSQSLLNSGDQKIYLTWYQQKPGQPPKLLIYWASTRESGVPDRFTGSVSGTDFTLTISSVQAEDLAVYYCQNDYNYPYTFGGGTKCCGGGGGVSRRRRRRGGRRRRLEIKRGSENLYFQGGSGKPIPNPLLGLDSTGGSGGSHHHHHH

SEQ ID NO: 79 - protein, 293 aa, Artificial Sequence
  fusion peptide
MAWVWTLLFLMAAAQSIQAEWIKQRPGQGLEWIGVIHPGNGGTNYNENFKGKATLTADKSSSTAYMQLSSLTSDDSAVYFCASGNDGSYWGQGTTVTVSSGGGGSGKGGSGGGGSGGGGSDIELTQSPSSLTVTAGEKVTMSCKSSQSLLNSGDQKIYLTWYQQKPGQPPKLLIYWASTRESGVPDRFTGSVSGTDFTLTISSVQAEDLAVYYCQNDYNYPYTFGGGTKCCGGGGGGKCSTRGRKCCRRKKLEIKRGSENLYFQGGSGKPIPNPLLGLDSTGGSGGSHHHHHH

SEQ ID NO: 80 - protein, 295 aa, Artificial Sequence
  fusion peptide
MAWVWTLLFLMAAAQSIQAEWIKQRPGQGLEWIGVIHPGNGGTNYNENFKGKATLTADKSSSTAYMQLSSLTSDDSAVYFCASGNDGSYWGQGTTVTVSSGGGGSGKGGSGGGGSGGGGSDIELTQSPSSLTVTAGEKVTMSCKSSQSLLNSGDQKIYLTWYQQKPGQPPKLLIYWASTRESGVPDRFTGSVSGTDFTLTISSVQAEDLAVYYCQNDYNYPYTFGGGTKCCGGGGGSSGGGGHRRCNKNNKKRLEIKRGSENLYFQGGSGKPIPNPLLGLDSTGGSGGSHHHHHH

SEQ ID NO: 81 - protein, 296 aa, Artificial Sequence
  fusion peptide
MAWVWTLLFLMAAAQSIQAEWIKQRPGQGLEWIGVIHPGNGGTNYNENFKGKATLTADKSSSTAYMQLSSLTSDDSAVYFCASGNDGSYWGQGTTVTVSSGGGGSGKGGSGGGGSGGGGSDIELTQSPSSLTVTAGEKVTMSCKSSQSLLNSGDQKIYLTWYQQKPGQPPKLLIYWASTRESGVPDRFTGSVSGTDFTLTISSVQAEDLAVYYCQNDYNYPYTFGGGTKCCGGGGGSSGGGGGRKKNNPNCRRHLEIKRGSENLYFQGGSGKPIPNPLLGLDSTGGSGGSHHHHHH

SEQ ID NO: 82 - protein, 301 aa, Artificial Sequence
  fusion peptide
MAWVWTLLFLMAAAQSIQAEWIKQRPGQGLEWIGVIHPGNGGTNYNENFKGKATLTADKSSSTAYMQLSSLTSDDSAVYFCASGNDGSYWGQGTTVTVSSGGGGSGKGGSGGGGSGGGGSDIELTQSPSSLTVTAGEKVTMSCKSSQSLLNSGDQKIYLTWYQQKPGQPPKLLIYWASTRESGVPDRFTGSVSGTDFTLTISSVQAEDLAVYYCQNDYNYPYTFGGGTKCCGGGGGSSGGGGGVSRRRRGGRRRRRRSVLEIKRGSENLYFQGGSGKPIPNPLLGLDSTGGSGGSHHHHHH

SEQ ID NO: 83 - protein, 300 aa, Artificial Sequence
  fusion peptide
MAWVWTLLFLMAAAQSIQAEWIKQRPGQGLEWIGVIHPGNGGTNYNENFKGKATLTADKSSSTAYMQLSSLTSDDSAVYFCASGNDGSYWGQGTTVTVSSGGGGSGKGGSGGGGSGGGGSDIELTQSPSSLTVTAGEKVTMSCKSSQSLLNSGDQKIYLTWYQQKPGQPPKLLIYWASTRESGVPDRFTGSVSGTDFTLTISSVQAEDLAVYYCQNDYNYPYTFGGGTKCCGGGGGSSGGGGGGKCSTRGRKCCRRKKLEIKRGSENLYFQGGSGKPIPNPLLGLDSTGGSGGSHHHHHH

SEQ ID NO: 84 - DNA, 34 bp, Artificial Sequence
  Primer
aaggagatatacatatgatggcatgggtttggac

SEQ ID NO: 85 - DNA, 46 bp, Artificial Sequence
  Primer
agcccgaagggaattcatttgcagatacaaagtgtttttagagttg

SEQ ID NO: 86 - protein, 11 aa, Artificial Sequence
  H4K
HRRCNKNNKKR

SEQ ID NO: 87 - protein, 11 aa, Artificial Sequence
  H4P
HRRCNPNNKKR

SEQ ID NO: 88 - protein, 14 aa, Artificial Sequence
  LMWP
VSRRRRRRGGRRRR

SEQ ID NO: 89 - protein, 15 aa, Artificial Sequence
  hBD3-3
GKCSTRGRKCCRRKK

SEQ ID NO: 90 - protein, 280 aa, Artificial Sequence
  fusion peptide
MAQVKLQESGPELVRPGTSVKVSCKASGYAFTNYLIEWIKQRPGQGLEWIGVIHPGNGGTNYNENFKGKATLTADKSSSTAYMQLSSLTSDDSAVYFCASGNDGSYWGQGTTVTVSSGGGGSGGGGSGGGGSDIELTQSPSSLTVTAGEKVTMSCKSSQSLLNSGDQKIYLTWYQQKPGQPPKLLIYWASTRESGVPDRFTGSVSGTDFTLTISSVQAEDLAVYYCQNDYNYPYTFGGGTKGGGGSGGGGSGGGGSHRRCNKNNKKRLEIKRLEHHHHHH

SEQ ID NO: 91 - protein, 280 aa, Artificial Sequence
  fusion peptide
MAQVKLQESGPELVRPGTSVKVSCKASGYAFTNYLIEWIKQRPGQGLEWIGVIHPGNGGTNYNENFKGKATLTADKSSSTAYMQLSSLTSDDSAVYFCASGNDGSYWGQGTTVTVSSGGGGSGGGGSGGGGSDIELTQSPSSLTVTAGEKVTMSCKSSQSLLNSGDQKIYLTWYQQKPGQPPKLLIYWASTRESGVPDRFTGSVSGTDFTLTISSVQAEDLAVYYCQNDYNYPYTFGGGTKGGGGSGGGGSGGGGSHRRCNPNNKKRLEIKRLEHHHHHH

SEQ ID NO: 92 - protein, 283 aa, Artificial Sequence
  fusion peptide
MAQVKLQESGPELVRPGTSVKVSCKASGYAFTNYLIEWIKQRPGQGLEWIGVIHPGNGGTNYNENFKGKATLTADKSSSTAYMQLSSLTSDDSAVYFCASGNDGSYWGQGTTVTVSSGGGGSGGGGSGGGGSDIELTQSPSSLTVTAGEKVTMSCKSSQSLLNSGDQKIYLTWYQQKPGQPPKLLIYWASTRESGVPDRFTGSVSGTDFTLTISSVQAEDLAVYYCQNDYNYPYTFGGGTKGGGGSGGGGSGGGGSVSRRRRRRGGRRRRLEIKRLEHHHHHH

SEQ ID NO: 93 - protein, 284 aa, Artificial Sequence
  fusion peptide
MAQVKLQESGPELVRPGTSVKVSCKASGYAFTNYLIEWIKQRPGQGLEWIGVIHPGNGGTNYNENFKGKATLTADKSSSTAYMQLSSLTSDDSAVYFCASGNDGSYWGQGTTVTVSSGGGGSGGGGSGGGGSDIELTQSPSSLTVTAGEKVTMSCKSSQSLLNSGDQKIYLTWYQQKPGQPPKLLIYWASTRESGVPDRFTGSVSGTDFTLTISSVQAEDLAVYYCQNDYNYPYTFGGGTKGGGGSGGGGSGGGGSGKCSTRGRKCCRRKKLEIKRLEHHHHHH